European Patent Application EP 4 137 145 A1, published February 22, 2023. Title: Pharmaceutical composition for treatment of neurodegenerative brain disease comprising glycine transporter as an active ingredient. Applicant: Amyloid Solution Inc Industry-Academic Cooperation Foundation, Yonsei University. The sequence listing filed with the application follows.

SEQUENCE LISTING (1 sequence)

SEQ ID NO: 1 - DNA, 1956 bp, Homo sapiens
atgagcggcggagacacgcgggctgcgatcgctcgccccaggatggccgcggctcatggacctgtggccccctcttccccagaacagaatggtgctgtgcccagcgaggccaccaagagggaccagaacctcaaacggggcaactggggcaaccagatcgagtttgtactgacgagcgtgggctatgccgtgggcctgggcaatgtctggcgcttcccatacctctgctatcgcaacgggggaggcgccttcatgttcccctacttcatcatgctcatcttctgcgggatccccctcttcttcatggagctctccttcggccagtttgcaagccaggggtgcctgggggtctggaggatcagccccatgttcaaaggagtgggctatggtatgatggtggtgtccacctacatcggcatctactacaatgtggtcatctgcatcgccttctactacttcttctcgtccatgacgcacgtgctgccctgggcctactgcaataacccctggaacacgcatgactgcgccggtgtactggacgcctccaacctcaccaatggctctcggccagccgccttgcccagcaacctctcccacctgctcaaccacagcctccagaggaccagccccagcgaggagtactggaggctgtacgtgctgaagctgtcagatgacattgggaactttggggaggtgcggctgcccctccttggctgcctcggtgtctcctggttggtcgtcttcctctgcctcatccgaggggtcaagtcttcagggaaagtggtgtacttcacggccacgttcccctacgtggtgctgaccattctgtttgtccgcggagtgaccctggagggagcctttgacggcatcatgtactacctaaccccgcagtgggacaagatcctggaggccaaggtgtggggtgatgctgcctcccagatcttctactcactgggctgcgcgtggggaggcctcatcaccatggcttcctacaacaagttccacaataactgttaccgggacagtgtcatcatcagcatcaccaactgtgccaccagcgtctatgctggcttcgtcatcttctccatcctcggcttcatggccaatcacctgggcgtggatgtgtcccgtgtggcagaccacggccctggcctggccttcgtggcttaccccgaggccctcacactacttcccatctccccgctgtggtctctgctcttcttcttcatgcttatcctgctggggctgggcactcagttctgcctcctggagacgctggtcacagccattgtggatgaggtggggaatgagtggatcctgcagaaaaagacctatgtgaccttgggcgtggctgtggctggcttcctgctgggcatccccctcaccagccaggcaggcatctattggctgctgctgatggacaactatgcggccagcttctccttggtggtcatctcctgcatcatgtgtgtggccatcatgtacatctacgggcaccggaactacttccaggacatccagatgatgctgggattcccaccacccctcttctttcagatctgctggcgcttcgtctctcccgccatcatcttctttattctagttttcactgtgatccagtaccagccgatcacctacaaccactaccagtacccaggctgggccgtggccattggcttcctcatggctctgtcctccgtcctctgcatccccctctacgccatgttccggctctgccgcacagacggggacaccctcctccagcgtttgaaaaatgccacaaagccaagcagagactggggccctgccctcctggagcaccggacagggcgctacgcccccaccatagccccctctcctgaggacggcttcgaggtccagccactgcacccggacaaggcgcagatccccattgtgggcagtaatggctccagccgcctccaggactcccggata